European Patent Specification EP 4 003 391 B1, published June 17, 2026. Title: PEPTIDES AND METHODS OF USING THE SAME. Applicant: SERPIN PHARMA, LLC. The sequence listing filed with the application follows.

SEQUENCE LISTING (46 sequences)

SEQ ID NO: 1 - protein, 9 aa, Homo sapiens
FNKPFVFLM

SEQ ID NO: 2 - protein, 17 aa, Homo sapiens
VKFNKPFVFLMIEQNTK

SEQ ID NO: 3 - protein, 5 aa, Homo sapiens
FVFLM

SEQ ID NO: 4 - protein, 9 aa, Artificial Sequence
  peptide derivative
  MISC_FEATURE (1)..(1): X=R or F
  MISC_FEATURE (3)..(3): X=K or R
  MISC_FEATURE (6)..(6): X=V or L
  MISC_FEATURE (7)..(7): X=F, V or I
  MISC_FEATURE (8)..(8): X=L, V or I
  MISC_FEATURE (9)..(9): X= M, I, or Nle
XNXPFXXXX

SEQ ID NO: 5 - protein, 9 aa, Artificial Sequence
  peptide derivative
  MOD_RES (9)..(9): Nle
FNKPFVFLX

SEQ ID NO: 6 - protein, 9 aa, Artificial Sequence
  peptide derivative
FNRPFLVVI

SEQ ID NO: 7 - protein, 9 aa, Artificial Sequence
  peptide derivative
  MOD_RES (9)..(9): Nle
FNRPFLVVX

SEQ ID NO: 8 - protein, 9 aa, Artificial Sequence
  peptide derivative
FNRPFLMII

SEQ ID NO: 9 - protein, 9 aa, Artificial Sequence
  peptide derivative
  MOD_RES (9)..(9): Nle
FNRPFLVIX

SEQ ID NO: 10 - protein, 5 aa, Artificial Sequence
  peptide derivative
  MOD_RES (5)..(5): Nle
FVFLX

SEQ ID NO: 11 - protein, 5 aa, Artificial Sequence
  peptide derivative
FLVVI

SEQ ID NO: 12 - protein, 5 aa, Artificial Sequence
  peptide derivative
  MOD_RES (5)..(5): Nle
FLVVX

SEQ ID NO: 13 - protein, 5 aa, Artificial Sequence
  peptide derivative
FLMII

SEQ ID NO: 14 - protein, 5 aa, Artificial Sequence
  peptide derivative
  MOD_RES (5)..(5): Nle
FLMIX

SEQ ID NO: 15 - protein, 5 aa, Artificial Sequence
  peptide derivative
  MISC_FEATURE (2)..(2): X=V or L
  MISC_FEATURE (3)..(3): X=F, V or M
  MISC_FEATURE (4)..(4): X= L, V or I
  MISC_FEATURE (5)..(5): X= M, I, or Nle
FXXXX

SEQ ID NO: 16 - protein, 31 aa, Artificial Sequence
  peptide derivative
  MISC_FEATURE (1)..(1): X=any basic amino acid or absent
  MISC_FEATURE (2)..(2): X=any basic amino acid or absent
  MISC_FEATURE (3)..(3): X=any basic amino acid or absent
  MISC_FEATURE (4)..(4): X=any basic amino acid or absent
  MISC_FEATURE (5)..(5): X=any basic amino acid or absent
  MISC_FEATURE (6)..(6): X=any basic amino acid or absent
  MISC_FEATURE (7)..(7): X=any basic amino acid or absent
  MISC_FEATURE (8)..(8): X=any basic amino acid or absent
  MISC_FEATURE (9)..(9): X=any basic amino acid or absent
  MISC_FEATURE (10)..(10): X=any basic amino acid
  MISC_FEATURE (12)..(12): X=R or F
  MISC_FEATURE (14)..(14): X=K or R
  MISC_FEATURE (17)..(17): X=V or L
  MISC_FEATURE (18)..(18): X=F, V or M
  MISC_FEATURE (19)..(19): X=L, V or I
  MISC_FEATURE (20)..(20): X=M, I, or Nle
  MISC_FEATURE (22)..(22): X=any basic amino acid
  MISC_FEATURE (23)..(23): X=any basic amino acid or absent
  MISC_FEATURE (24)..(24): X=any basic amino acid or absent
  MISC_FEATURE (25)..(25): X=any basic amino acid or absent
  MISC_FEATURE (26)..(26): X=any basic amino acid or absent
  MISC_FEATURE (27)..(27): X=any basic amino acid or absent
  MISC_FEATURE (28)..(28): X=any basic amino acid or absent
  MISC_FEATURE (29)..(29): X=any basic amino acid or absent
  MISC_FEATURE (30)..(30): X=any basic amino acid or absent
  MISC_FEATURE (31)..(31): X=any basic amino acid or absent
XXXXXXXXXXRXNXPFXXXXRXXXXXXXXXX

SEQ ID NO: 17 - protein, 31 aa, Artificial Sequence
  peptide derivative
  MISC_FEATURE (1)..(1): X=any basic amino acid or absent
  MISC_FEATURE (2)..(2): X=any basic amino acid or absent
  MISC_FEATURE (3)..(3): X=any basic amino acid or absent
  MISC_FEATURE (4)..(4): X=any basic amino acid or absent
  MISC_FEATURE (5)..(5): X=any basic amino acid or absent
  MISC_FEATURE (6)..(6): X=any basic amino acid or absent
  MISC_FEATURE (7)..(7): X=any basic amino acid or absent
  MISC_FEATURE (8)..(8): X=any basic amino acid or absent
  MISC_FEATURE (9)..(9): X=any basic amino acid or absent
  MISC_FEATURE (10)..(10): X=any basic amino acid
  MISC_FEATURE (22)..(22): X=any basic amino acid
  MISC_FEATURE (23)..(23): X=any basic amino acid or absent
  MISC_FEATURE (24)..(24): X=any basic amino acid or absent
  MISC_FEATURE (25)..(25): X=any basic amino acid or absent
  MISC_FEATURE (26)..(26): X=any basic amino acid or absent
  MISC_FEATURE (27)..(27): X=any basic amino acid or absent
  MISC_FEATURE (28)..(28): X=any basic amino acid or absent
  MISC_FEATURE (29)..(29): X=any basic amino acid or absent
  MISC_FEATURE (30)..(30): X=any basic amino acid or absent
  MISC_FEATURE (31)..(31): X=any basic amino acid or absent
XXXXXXXXXXRFNRPFLVVIRXXXXXXXXXX

SEQ ID NO: 18 - protein, 31 aa, Artificial Sequence
  peptide derivative
  MISC_FEATURE (1)..(1): X=any basic amino acid or absent
  MISC_FEATURE (2)..(2): X=any basic amino acid or absent
  MISC_FEATURE (3)..(3): X=any basic amino acid or absent
  MISC_FEATURE (4)..(4): X=any basic amino acid or absent
  MISC_FEATURE (5)..(5): X=any basic amino acid or absent
  MISC_FEATURE (6)..(6): X=any basic amino acid or absent
  MISC_FEATURE (7)..(7): X=any basic amino acid or absent
  MISC_FEATURE (8)..(8): X=any basic amino acid or absent
  MISC_FEATURE (9)..(9): X=any basic amino acid or absent
  MISC_FEATURE (10)..(10): X=any basic amino acid
  MISC_FEATURE (22)..(22): X= any basic amino acid
  MISC_FEATURE (23)..(23): X= any basic amino acid or absent
  MISC_FEATURE (24)..(24): X= any basic amino acid or absent
  MISC_FEATURE (25)..(25): X= any basic amino acid or absent
  MISC_FEATURE (26)..(26): X= any basic amino acid or absent
  MISC_FEATURE (27)..(27): X= any basic amino acid or absent
  MISC_FEATURE (28)..(28): X= any basic amino acid or absent
  MISC_FEATURE (29)..(29): X= any basic amino acid or absent
  MISC_FEATURE (30)..(30): X= any basic amino acid or absent
  MISC_FEATURE (31)..(31): X= any basic amino acid or absent
XXXXXXXXXXRFNRPFLMIIRXXXXXXXXXX

SEQ ID NO: 19 - protein, 31 aa, Artificial Sequence
  peptide derivative
  MISC_FEATURE (1)..(1): X=any basic amino acid or absent
  MISC_FEATURE (2)..(2): X=any basic amino acid or absent
  MISC_FEATURE (3)..(3): X=any basic amino acid or absent
  MISC_FEATURE (4)..(4): X=any basic amino acid or absent
  MISC_FEATURE (5)..(5): X=any basic amino acid or absent
  MISC_FEATURE (6)..(6): X=any basic amino acid or absent
  MISC_FEATURE (7)..(7): X=any basic amino acid or absent
  MISC_FEATURE (8)..(8): X=any basic amino acid or absent
  MISC_FEATURE (9)..(9): X=any basic amino acid or absent
  MISC_FEATURE (10)..(10): X=any basic amino acid
  MOD_RES (20)..(20): Nle
  MISC_FEATURE (22)..(22): X=any basic amino acid
  MISC_FEATURE (23)..(23): X=any basic amino acid or absent
  MISC_FEATURE (24)..(24): X=any basic amino acid or absent
  MISC_FEATURE (25)..(25): X=any basic amino acid or absent
  MISC_FEATURE (26)..(26): X=any basic amino acid or absent
  MISC_FEATURE (27)..(27): X=any basic amino acid or absent
  MISC_FEATURE (28)..(28): X=any basic amino acid or absent
  MISC_FEATURE (29)..(29): X=any basic amino acid or absent
  MISC_FEATURE (30)..(30): X=any basic amino acid or absent
  MISC_FEATURE (31)..(31): X=any basic amino acid or absent
XXXXXXXXXXKFNKPFVFLXRXXXXXXXXXX

SEQ ID NO: 20 - protein, 16 aa, Artificial Sequence
  peptide derivative
  MISC_FEATURE (1)..(1): X=V or L
  MISC_FEATURE (2)..(2): X=any amino acid
  MISC_FEATURE (3)..(3): X=R or F
  MISC_FEATURE (4)..(4): X=any amino acid
  MISC_FEATURE (5)..(5): X=R or K
  MISC_FEATURE (6)..(6): X=any amino acid
  MISC_FEATURE (11)..(11): X=M, Nle, or I
  MISC_FEATURE (12)..(12): X=any amino acid
  MISC_FEATURE (13)..(13): X=any amino acid
  MISC_FEATURE (14)..(14): X=any amino acid
  MISC_FEATURE (15)..(15): X=any amino acid
  MISC_FEATURE (16)..(16): X=any amino acid
XXXXXXFVFLXXXXXX

SEQ ID NO: 21 - protein, 17 aa, Artificial Sequence
  peptide derivative
  MISC_FEATURE (1)..(1): X=V or L
  MISC_FEATURE (2)..(2): X=any amino acid
  MISC_FEATURE (3)..(3): X=F or R
  MISC_FEATURE (4)..(4): X=any amino acid
  MISC_FEATURE (5)..(5): X=any amino acid
  MISC_FEATURE (6)..(6): X=K or R
  MISC_FEATURE (7)..(7): X=any amino acid
  MISC_FEATURE (9)..(9): X=V, L, or M
  MISC_FEATURE (12)..(12): X=M, Nle, or I
  MISC_FEATURE (13)..(13): X=any amino acid
  MISC_FEATURE (14)..(14): X=any amino acid
  MISC_FEATURE (15)..(15): X=any amino acid
  MISC_FEATURE (16)..(16): X=any amino acid
  MISC_FEATURE (17)..(17): X=any amino acid
XXXXXXXFXFLXXXXXX

SEQ ID NO: 22 - protein, 21 aa, Artificial Sequence
  peptide derivative
FPKMVPQFNTELKIFPEVNIK

SEQ ID NO: 23 - protein, 33 aa, Homo sapiens
SIPPEVKFNKPFVFLMIEQNTKSPLFMGKVVNP

SEQ ID NO: 24 - protein, 17 aa, Homo sapiens
VKFNKPFVFLMIEQNTK

SEQ ID NO: 25 - protein, 11 aa, Homo sapiens
VKFNKPFVFLM

SEQ ID NO: 26 - protein, 23 aa, Artificial Sequence
  peptide derivative
RRRVKFNKPFVFLMIEQNTKRRR

SEQ ID NO: 27 - protein, 17 aa, Artificial Sequence
  peptide derivative
RRRVKFNKPFVFLMRRR

SEQ ID NO: 28 - protein, 17 aa, Artificial Sequence
  peptide derivative
LRFNRPFLVVIFSTSTQ

SEQ ID NO: 29 - protein, 11 aa, Artificial Sequence
  peptide derivative
LRFNRPFLVVI

SEQ ID NO: 30 - protein, 17 aa, Artificial Sequence
  peptide derivative
RRRLRFNRPFLVVIRRR

SEQ ID NO: 31 - protein, 11 aa, Artificial Sequence
  peptide derivative
VRFNRPFLMII

SEQ ID NO: 32 - protein, 17 aa, Artificial Sequence
  peptide derivative
RRRVRFNRPFLMIIRRR

SEQ ID NO: 33 - protein, 8 aa, Artificial Sequence
  peptide derivative
VRFNRPFL

SEQ ID NO: 34 - protein, 14 aa, Artificial Sequence
  peptide derivative
RRRVRFNRPFLRRR

SEQ ID NO: 35 - protein, 17 aa, Artificial Sequence
  peptide derivative
  MOD_RES (11)..(11): Nle
VKFNKPFVFLXIEQNTK

SEQ ID NO: 36 - protein, 17 aa, Artificial Sequence
  peptide derivative
VKFNKAAAAAAIEQNTK

SEQ ID NO: 37 - protein, 31 aa, Artificial Sequence
  peptide derivative
  MISC_FEATURE (1)..(1): X=any amino acid or absent
  MISC_FEATURE (2)..(2): X=any amino acid or absent
  MISC_FEATURE (3)..(3): X=any amino acid or absent
  MISC_FEATURE (4)..(4): X=any amino acid or absent
  MISC_FEATURE (5)..(5): X=any amino acid or absent
  MISC_FEATURE (6)..(6): X=any amino acid or absent
  MISC_FEATURE (7)..(7): X=any amino acid or absent
  MISC_FEATURE (8)..(8): X=any amino acid or absent
  MISC_FEATURE (9)..(9): X=any amino acid or absent
  MISC_FEATURE (10)..(10): X=any amino acid
  MOD_RES (20)..(20): Nle
  MISC_FEATURE (22)..(22): X=any amino acid or absent
  MISC_FEATURE (23)..(23): X=any amino acid or absent
  MISC_FEATURE (24)..(24): X=any amino acid or absent
  MISC_FEATURE (25)..(25): X=any amino acid or absent
  MISC_FEATURE (26)..(26): X=any amino acid or absent
  MISC_FEATURE (27)..(27): X=any amino acid or absent
  MISC_FEATURE (28)..(28): X=any amino acid or absent
  MISC_FEATURE (29)..(29): X=any amino acid or absent
  MISC_FEATURE (30)..(30): X=any amino acid or absent
  MISC_FEATURE (31)..(31): X=any amino acid or absent
XXXXXXXXXXRFNKPFVFLXRXXXXXXXXXX

SEQ ID NO: 38 - protein, 11 aa, Artificial Sequence
  peptide derivative
VKFNKPFVFLM

SEQ ID NO: 39 - protein, 11 aa, Artificial Sequence
  peptide derivative
LRFNRPFLVVI

SEQ ID NO: 40 - protein, 11 aa, Artificial Sequence
  peptide derivative
  MOD_RES (11)..(11): Nle
VKFNKPFVFLX

SEQ ID NO: 41 - protein, 11 aa, Artificial Sequence
  peptide derivative
RFNRPFLVVIR

SEQ ID NO: 42 - protein, 11 aa, Artificial Sequence
  peptide derivative
RFNRPFLMIIR

SEQ ID NO: 43 - protein, 11 aa, Artificial Sequence
  peptide derivative
  MOD_RES (10)..(10): Nle
RFNKPFVFLXR

SEQ ID NO: 44 - protein, 11 aa, Artificial Sequence
  peptide derivative
RRRFLVVIRRR

SEQ ID NO: 45 - protein, 11 aa, Artificial Sequence
  peptide derivative
RRRFLMIIRRR

SEQ ID NO: 46 - protein, 11 aa, Artificial Sequence
  peptide derivative
  MOD_RES (8)..(8): Nle
RRRFVFLXRRR